European Patent Application EP 4 410 834 A1, published August 7, 2024. Title: CTLA-4结合分子及其应用. Applicant: 浙江纳米抗体技术中心有限公司. Application CN. The sequence listing filed with the application follows.

SEQUENCE LISTING (80 sequences)

SEQ ID NO: 1-3 - skipped (3 entries)

SEQ ID NO: 4 - protein, 8 aa, synthetic construct
  REGION 1..8: note = CDR1
GSTLDPFV

SEQ ID NO: 5 - protein, 8 aa, synthetic construct
  REGION 1..8: note = CDR1
GLNFGIYD

SEQ ID NO: 6 - protein, 8 aa, synthetic construct
  REGION 1..8: note = CDR1
GDTLESFA

SEQ ID NO: 7 - protein, 8 aa, synthetic construct
  REGION 1..8: note = CDR1
GFTLDDHA

SEQ ID NO: 8 - protein, 8 aa, synthetic construct
  REGION 1..8: note = CDR1
GFSSDYYD

SEQ ID NO: 9 - protein, 8 aa, synthetic construct
  REGION 1..8: note = CDR1
GFTLDDQA

SEQ ID NO: 10 - protein, 8 aa, synthetic construct
  REGION 1..8: note = CDR1
GGTLDYWS

SEQ ID NO: 11 - protein, 6 aa, synthetic construct
  REGION 1..6: note = CDR2
INRSRT

SEQ ID NO: 12 - protein, 6 aa, synthetic construct
  REGION 1..6: note = CDR2
INRNRA

SEQ ID NO: 13 - protein, 8 aa, synthetic construct
  REGION 1..8: note = CDR2
MNPDGDIT

SEQ ID NO: 14 - protein, 8 aa, synthetic construct
  REGION 1..8: note = CDR2
IGRTGEFT

SEQ ID NO: 15 - protein, 7 aa, synthetic construct
  REGION 1..7: note = CDR2
ISSSGRT

SEQ ID NO: 16 - protein, 8 aa, synthetic construct
  REGION 1..8: note = CDR2
IRSSGGST

SEQ ID NO: 17 - protein, 7 aa, synthetic construct
  REGION 1..7: note = CDR2
ISSSGRG

SEQ ID NO: 18 - protein, 8 aa, synthetic construct
  REGION 1..8: note = CDR2
ISGTGLRT

SEQ ID NO: 19 - protein, 22 aa, synthetic construct
  REGION 1..22: note = CDR3
AASPDKPFYTDQTMCNKHYYGY

SEQ ID NO: 20 - protein, 22 aa, synthetic construct
  REGION 1..22: note = CDR3
AASPDKAFYTDQTMCNIHYYGY

SEQ ID NO: 21 - protein, 13 aa, synthetic construct
  REGION 1..13: note = CDR3
ALGPERYFSIYAT

SEQ ID NO: 22 - protein, 19 aa, synthetic construct
  REGION 1..19: note = CDR3
AAERLVFHLCSLSEYDYDT

SEQ ID NO: 23 - protein, 19 aa, synthetic construct
  REGION 1..19: note = CDR3
ASVPTLGTACLMTHGMRSD

SEQ ID NO: 24 - protein, 19 aa, synthetic construct
  REGION 1..19: note = CDR3
GLAPISPVHAVCNQHYFGY

SEQ ID NO: 25 - protein, 19 aa, synthetic construct
  REGION 1..19: note = CDR3
ASVPAVQTMCLMTHASRDD

SEQ ID NO: 26 - protein, 19 aa, synthetic construct
  REGION 1..19: note = CDR3
TGKLLHPSLWSACANEYDL

SEQ ID NO: 27 - protein, 127 aa, synthetic construct
  REGION 1..127: note = amino acid sequence of antibody
EVQLVESGGGLAQPGGSLRLSCAASGSTLDPFVIGWFRQAPGKERETVACINRSRTSYADSVKGRFTISRDNAKNMVYLQMNSLKPEDTAVYYCAASPDKPFYTDQTMCNKHYYGYWTQGTQVTVSS

SEQ ID NO: 28 - protein, 127 aa, synthetic construct
  REGION 1..127: note = amino acid sequence of antibody
EVQLVESGGGLAQSGGSLRLSCAVSGSTLDPFVIGWFRQAPGKERETVSCINRNRASYADGVKGRFTISRDTAKNMVYLQMNSLKPEDTAVYYCAASPDKAFYTDQTMCNIHYYGYWAQGTQVTVSS

SEQ ID NO: 29 - protein, 127 aa, synthetic construct
  REGION 1..127: note = amino acid sequence of antibody
QVQLVESGGGLAQSGGSLRLSCAVSGSTLDPFVIGWFRQAPGKERETVSCINRNRASYADGVKGRFTISRDTAKNMVYLQMNSLKPEDTAVYYCAASPDKAFYTDQTMCNIHYYGYWAQGTLVTVSS

SEQ ID NO: 30 - protein, 120 aa, synthetic construct
  REGION 1..120: note = amino acid sequence of antibody
EVQLVESGGGLVQPGGSLRLSCAVSGLNFGIYDFTWGRQAPGKGLEWIATMNPDGDITNYVDSVKGRFTISRDNANESLYLQMNSLKPEDTALYYCALGPERYFSIYATRGQGTLVTVSS

SEQ ID NO: 31 - protein, 126 aa, synthetic construct
  REGION 1..126: note = amino acid sequence of antibody
QVQLVESGGGLVQPGGSLRLSCASSGDTLESFAVGWFRQAPGKEREELACIGRTGEFTDYPGSVKGRFTITRDNAKNTVYLEMVNLKAEDTGVYYCAAERLVFHLCSLSEYDYDTWGQGTQVTVSS

SEQ ID NO: 32 - protein, 125 aa, synthetic construct
  REGION 1..125: note = amino acid sequence of antibody
EVQLVESGGGLVQPGGSLRLSCVASGFTLDDHAIGWFRQAPGKAREGVSCISSSGRTTYLLSVKGRFTITRDNAKNTAYLQMNRLQPEDTAVYYCASVPTLGTACLMTHGMRSDWGQGTQVTVSS

SEQ ID NO: 33 - protein, 126 aa, synthetic construct
  REGION 1..126: note = amino acid sequence of antibody
QVQLVESGGGLVQPGGSLRLSCAVSGFSSDYYDIGWFRQDPEKEREMVSCIRSSGGSTKYADSVKGRFTISRDNAKNTVYLQMNSLEPEDTAVYYCGLAPISPVHAVCNQHYFGYWGQGTRVTVSS

SEQ ID NO: 34 - protein, 125 aa, synthetic construct
  REGION 1..125: note = amino acid sequence of antibody
QVQLVESGGGLVQPGGSLRLSCAASGFTLDDQAIGWFRQAPGKEREGVACISSSGRGTYLLSVKGRFTVTRDNAKNTVYLQMNRLQPEDTAVYYCASVPAVQTMCLMTHASRDDWGQGTQVTVSS

SEQ ID NO: 35 - protein, 126 aa, synthetic construct
  REGION 1..126: note = amino acid sequence of antibody
QVQLVESGGGLVQPGGSLRLSCEASGGTLDYWSIGWFRQAPGKEREEVSCISGTGLRTNYADSVKGRFTVSRDNSRNSVILQMNSLKPEDTGVYYCTGKLLHPSLWSACANEYDLWGQGTQVTVSS

SEQ ID NO: 36 - protein, 126 aa, synthetic construct
  REGION 1..126: note = amino acid sequence of antibody
EVQLVESGGGLVQPGGSLRLSCAASGFSSDYYDIGWFRQAPGKEREMVSCIRSSGGSTKYADSVKGRFTISRDNSKNTVYLQMNSLRAEDTAVYYCGLAPISPVHAVCNQHYFGYWGQGTRVTVSS

SEQ ID NO: 37 - protein, 126 aa, synthetic construct
  REGION 1..126: note = amino acid sequence of antibody
EVQLVESGGGLVQPGGSLRLSCAASGFSSDYYDIGWFRQDPGKEREMVSCIRSSGGSTKYADSVKGRFTISRDNSKNTVYLQMNSLRAEDTAVYYCGLAPISPVHAVCNQHYFGYWGQGTRVTVSS

SEQ ID NO: 38 - protein, 126 aa, synthetic construct
  REGION 1..126: note = amino acid sequence of antibody
EVQLVESGGGLVQPGGSLRLSCAASGFSSDYYDIGWFRQAPEKEREMVSCIRSSGGSTKYADSVKGRFTISRDNSKNTVYLQMNSLRAEDTAVYYCGLAPISPVHAVCNQHYFGYWGQGTRVTVSS

SEQ ID NO: 39 - protein, 126 aa, synthetic construct
  REGION 1..126: note = amino acid sequence of antibody
EVQLVESGGGLVQPGGSLRLSCAASGFSSDYYDIGWFRQDPEKEREMVSCIRSSGGSTKYADSVKGRFTISRDNSKNTVYLQMNSLRAEDTAVYYCGLAPISPVHAVCNQHYFGYWGQGTRVTVSS

SEQ ID NO: 40 - protein, 126 aa, synthetic construct
  REGION 1..126: note = amino acid sequence of antibody
EVQLVESGGGLVQPGGSLRLSCAASGFSSDYYDIGWFRQDPEKEREMVSCIRSSGGSTKYADSVKGRFTISRDNSKNTVYLQMNSLEAEDTAVYYCGLAPISPVHAVCNQHYFGYWGQGTRVTVSS

SEQ ID NO: 41 - protein, 126 aa, synthetic construct
  REGION 1..126: note = amino acid sequence of antibody
EVQLVESGGGLVQPGGSLRLSCAASGGTLDYWSIGWFRQAPGKEREEVSCISGTGLRTNYADSVKGRFTISRDNSKNTVYLQMNSLRAEDTAVYYCTGKLLHPSLWSACANEYDLWGQGTQVTVSS

SEQ ID NO: 42 - protein, 126 aa, synthetic construct
  REGION 1..126: note = amino acid sequence of antibody
EVQLVESGGGLVQPGGSLRLSCAASGGTLDYWSIGWFRQAPGKEREEVSCISGTGLRTNYADSVKGRFTISRDNSKNTVILQMNSLRAEDTAVYYCTGKLLHPSLWSACANEYDLWGQGTQVTVSS

SEQ ID NO: 43 - protein, 126 aa, synthetic construct
  REGION 1..126: note = amino acid sequence of antibody
EVQLVESGGGLVQPGGSLRLSCAASGGTLDYWSIGWFRQAPGKEREEVSCISGTGLRTNYADSVKGRFTISRDNSKNTVYLQMNSLRAEDTGVYYCTGKLLHPSLWSACANEYDLWGQGTQVTVSS

SEQ ID NO: 44 - protein, 126 aa, synthetic construct
  REGION 1..126: note = amino acid sequence of antibody
EVQLVESGGGLVQPGGSLRLSCAASGGTLDYWSIGWFRQAPGKEREEVSCISGTGLRTNYADSVKGRFTISRDNSKNTVILQMNSLRAEDTGVYYCTGKLLHPSLWSACANEYDLWGQGTQVTVSS

SEQ ID NO: 45 - protein, 126 aa, synthetic construct
  REGION 1..126: note = amino acid sequence of antibody
EVQLVESGGGLVQPGGSLRLSCAASGGTLDYWSIGWFRQAPGKEREEVSCISGTGLRTNYADSVKGRFTVSRDNSKNTVILQMNSLRAEDTGVYYCTGKLLHPSLWSACANEYDLWGQGTQVTVSS

SEQ ID NO: 46 - protein, 126 aa, synthetic construct
  REGION 1..126: note = amino acid sequence of antibody
EVQLVESGGGLVQPGGSLRLSCAASGGTLDYWSIGWFRQAPGKEREEVSCISGTGLRTNYADSVKGRFTVSRDNSKNSVILQMNSLRAEDTGVYYCTGKLLHPSLWSACANEYDLWGQGTQVTVSS

SEQ ID NO: 47 - protein, 126 aa, synthetic construct
  REGION 1..126: note = amino acid sequence of antibody
EVQLVESGGGLVQPGGSLRLSCEASGGTLDYWSIGWFRQAPGKEREEVSCISGTGLRTNYADSVKGRFTISRDNSKNTVYLQMNSLRAEDTAVYYCTGKLLHPSLWSACANEYDLWGQGTQVTVSS

SEQ ID NO: 48 - protein, 126 aa, synthetic construct
  REGION 1..126: note = amino acid sequence of antibody
EVQLVESGGGLVQPGGSLRLSCEASGGTLDYWSIGWFRQAPGKEREEVSCISGTGLRTNYADSVKGRFTISRDNSKNTVILQMNSLRAEDTAVYYCTGKLLHPSLWSACANEYDLWGQGTQVTVSS

SEQ ID NO: 49 - protein, 126 aa, synthetic construct
  REGION 1..126: note = amino acid sequence of antibody
EVQLVESGGGLVQPGGSLRLSCEASGGTLDYWSIGWFRQAPGKEREEVSCISGTGLRTNYADSVKGRFTISRDNSKNTVYLQMNSLRAEDTGVYYCTGKLLHPSLWSACANEYDLWGQGTQVTVSS

SEQ ID NO: 50 - protein, 126 aa, synthetic construct
  REGION 1..126: note = amino acid sequence of antibody
EVQLVESGGGLVQPGGSLRLSCEASGGTLDYWSIGWFRQAPGKEREEVSCISGTGLRTNYADSVKGRFTISRDNSKNTVILQMNSLRAEDTGVYYCTGKLLHPSLWSACANEYDLWGQGTQVTVSS

SEQ ID NO: 51 - protein, 126 aa, synthetic construct
  REGION 1..126: note = amino acid sequence of antibody
EVQLVESGGGLVQPGGSLRLSCEASGGTLDYWSIGWFRQAPGKEREEVSCISGTGLRTNYADSVKGRFTVSRDNSKNTVILQMNSLRAEDTGVYYCTGKLLHPSLWSACANEYDLWGQGTQVTVSS

SEQ ID NO: 52 - protein, 127 aa, synthetic construct
  REGION 1..127: note = amino acid sequence of antibody
EVQLVESGGGLVQPGGSLRLSCAASGSTLDPFVIGWFRQAPGKERETVSCINRSRTSYADSVKGRFTISRDNSKNTVYLQMNSLRAEDTAVYYCAASPDKPFYTDQTMCNKHYYGYWTQGTQVTVSS

SEQ ID NO: 53 - protein, 127 aa, synthetic construct
  REGION 1..127: note = amino acid sequence of antibody
EVQLVESGGGLVQPGGSLRLSCAASGSTLDPFVIGWFRQAPGKERETVSCINRSRTSYADSVKGRFTISRDNSKNMVYLQMNSLRAEDTAVYYCAASPDKPFYTDQTMCNKHYYGYWTQGTQVTVSS

SEQ ID NO: 54 - protein, 127 aa, synthetic construct
  REGION 1..127: note = amino acid sequence of antibody
EVQLVESGGGLVQPGGSLRLSCAASGSTLDPFVIGWFRQAPGKERETVSCINRSRTSYADSVKGRFTISRDNAKNTVYLQMNSLRAEDTAVYYCAASPDKPFYTDQTMCNKHYYGYWTQGTQVTVSS

SEQ ID NO: 55 - protein, 127 aa, synthetic construct
  REGION 1..127: note = amino acid sequence of antibody
EVQLVESGGGLVQPGGSLRLSCAASGSTLDPFVIGWFRQAPGKERETVACINRSRTSYADSVKGRFTISRDNSKNTVYLQMNSLRAEDTAVYYCAASPDKPFYTDQTMCNKHYYGYWTQGTQVTVSS

SEQ ID NO: 56 - protein, 127 aa, synthetic construct
  REGION 1..127: note = amino acid sequence of antibody
EVQLVESGGGLVQPGGSLRLSCAASGSTLDPFVIGWFRQAPGKERETVACINRSRTSYADSVKGRFTISRDNSKNMVYLQMNSLRAEDTAVYYCAASPDKPFYTDQTMCNKHYYGYWTQGTQVTVSS

SEQ ID NO: 57 - protein, 127 aa, synthetic construct
  REGION 1..127: note = amino acid sequence of antibody
EVQLVESGGGLVQPGGSLRLSCAASGSTLDPFVIGWFRQAPGKERETVACINRSRTSYADSVKGRFTISRDNAKNTVYLQMNSLRAEDTAVYYCAASPDKPFYTDQTMCNKHYYGYWTQGTQVTVSS

SEQ ID NO: 58 - protein, 127 aa, synthetic construct
  REGION 1..127: note = amino acid sequence of antibody
EVQLVESGGGLVQPGGSLRLSCAASGSTLDPFVIGWFRQAPGKERETVACINRSRTSYADSVKGRFTISRDNAKNMVYLQMNSLRAEDTAVYYCAASPDKPFYTDQTMCNKHYYGYWTQGTQVTVSS

SEQ ID NO: 59 - protein, 127 aa, synthetic construct
  REGION 1..127: note = amino acid sequence of antibody
EVQLVESGGGLVQPGGSLRLSCAASGSTLDPFVIGWFRQAPGKERETVSCINRSRTSYADSVKGRFTISRDNSKNTLYLQMNSLRAEDTAVYYCAASPDKPFYTDQTMCNKHYYGYWTQGTQVTVSS

SEQ ID NO: 60 - protein, 127 aa, synthetic construct
  REGION 1..127: note = amino acid sequence of antibody
EVQLVESGGGLVQPGGSLRLSCAASGSTLDPFVIGWFRQAPGKGRETVACINRSRTSYADSVKGRFTISRDNAKNMVYLQMNSLRAEDTAVYYCAASPDKPFYTDQTMCNKHYYGYWTQGTQVTVSS

SEQ ID NO: 61 - protein, 127 aa, synthetic construct
  REGION 1..127: note = amino acid sequence of antibody
EVQLVESGGGLVQPGGSLRLSCAASGSTLDPFVIGWFRQAPGKGRETVSCINRSRTSYADSVKGRFTISRDNSKNTVYLQMNSLRAEDTAVYYCAASPDKPFYTDQTMCNKHYYGYWTQGTQVTVSS

SEQ ID NO: 62 - protein, 126 aa, synthetic construct
  REGION 1..126: note = amino acid sequence of antibody
EVQLVESGGGLVQPGGSLRLSCAASGDTLESFAVGWFRQAPGKEREELSCIGRTGEFTDYPGSVKGRFTISRDNSKNTVYLQMNSLRAEDTAVYYCAAERLVFHLCSLSEYDYDTWGQGTQVTVSS

SEQ ID NO: 63 - protein, 126 aa, synthetic construct
  REGION 1..126: note = amino acid sequence of antibody
EVQLVESGGGLVQPGGSLRLSCAASGDTLESFAVGWFRQAPGKEREELSCIGRTGEFTDYPGSVKGRFTISRDNAKNTVYLQMNSLRAEDTAVYYCAAERLVFHLCSLSEYDYDTWGQGTQVTVSS

SEQ ID NO: 64 - protein, 126 aa, synthetic construct
  REGION 1..126: note = amino acid sequence of antibody
EVQLVESGGGLVQPGGSLRLSCAASGDTLESFAVGWFRQAPGKEREELSCIGRTGEFTDYPGSVKGRFTITRDNSKNTVYLQMNSLRAEDTAVYYCAAERLVFHLCSLSEYDYDTWGQGTQVTVSS

SEQ ID NO: 65 - protein, 126 aa, synthetic construct
  REGION 1..126: note = amino acid sequence of antibody
EVQLVESGGGLVQPGGSLRLSCAASGDTLESFAVGWFRQAPGKEREELACIGRTGEFTDYPGSVKGRFTISRDNSKNTVYLQMNSLRAEDTAVYYCAAERLVFHLCSLSEYDYDTWGQGTQVTVSS

SEQ ID NO: 66 - protein, 126 aa, synthetic construct
  REGION 1..126: note = amino acid sequence of antibody
EVQLVESGGGLVQPGGSLRLSCAASGDTLESFAVGWFRQAPGKEREELACIGRTGEFTDYPGSVKGRFTISRDNAKNTVYLQMNSLRAEDTAVYYCAAERLVFHLCSLSEYDYDTWGQGTQVTVSS

SEQ ID NO: 67 - protein, 126 aa, synthetic construct
  REGION 1..126: note = amino acid sequence of antibody
EVQLVESGGGLVQPGGSLRLSCAASGDTLESFAVGWFRQAPGKEREELACIGRTGEFTDYPGSVKGRFTITRDNSKNTVYLQMNSLRAEDTAVYYCAAERLVFHLCSLSEYDYDTWGQGTQVTVSS

SEQ ID NO: 68 - protein, 126 aa, synthetic construct
  REGION 1..126: note = amino acid sequence of antibody
EVQLVESGGGLVQPGGSLRLSCAASGDTLESFAVGWFRQAPGKEREELACIGRTGEFTDYPGSVKGRFTITRDNAKNTVYLQMNSLRAEDTAVYYCAAERLVFHLCSLSEYDYDTWGQGTQVTVSS

SEQ ID NO: 69 - protein, 126 aa, synthetic construct
  REGION 1..126: note = amino acid sequence of antibody
EVQLVESGGGLVQPGGSLRLSCAASGDTLESFAVGWFRQAPGKEREEVACIGRTGEFTDYPGSVKGRFTISRDNSKNTVYLQMNSLRAEDTAVYYCAAERLVFHLCSLSEYDYDTWGQGTQVTVSS

SEQ ID NO: 70 - protein, 126 aa, synthetic construct
  REGION 1..126: note = amino acid sequence of antibody
EVQLVESGGGLVQPGGSLRLSCAASGDTLESFAVGWFRQAPGKEREEVACIGRTGEFTDYPGSVKGRFTISRDNAKNTVYLQMNSLRAEDTAVYYCAAERLVFHLCSLSEYDYDTWGQGTQVTVSS

SEQ ID NO: 71 - protein, 126 aa, synthetic construct
  REGION 1..126: note = amino acid sequence of antibody
EVQLVESGGGLVQPGGSLRLSCAASGDTLESFAVGWFRQAPGKEREEVACIGRTGEFTDYPGSVKGRFTITRDNSKNTVYLQMNSLRAEDTAVYYCAAERLVFHLCSLSEYDYDTWGQGTQVTVSS

SEQ ID NO: 72 - protein, 126 aa, synthetic construct
  REGION 1..126: note = amino acid sequence of antibody
EVQLVESGGGLVQPGGSLRLSCAASGDTLESFAVGWFRQAPGKEREELACIGRTGEFTDYPGSVKGRFTITRDNSKNTVYLEMNSLRAEDTAVYYCAAERLVFHLCSLSEYDYDTWGQGTQVTVSS

SEQ ID NO: 73 - protein, 126 aa, synthetic construct
  REGION 1..126: note = amino acid sequence of antibody
EVQLVESGGGLVQPGGSLRLSCASSGDTLESFAVGWFRQAPGKEREELACIGRTGEFTDYPGSVKGRFTITRDNSKNTVYLQMVSLRAEDTAVYYCAAERLVFHLCSLSEYDYDTWGQGTQVTVSS

SEQ ID NO: 74 - protein, 229 aa, synthetic construct
  REGION 1..229: note = amino acid sequence of antibody
ESKYGPPCPPCPAPEFLGGPSVFLFPPKPKDTLMISRTPEVTCVVVDVSQEDPEVQFNWYVDGVEVHNAKTKPREEQFNSTYRVVSVLTVLHQDWLNGKEYKCKVSNKGLPSSIEKTISKAKGQPREPQVYTLPPSQEEMTKNQVSLTCLVKGFYPSDIAVEWESNGQPENNYKTTPPVLDSDGSFFLYSRLTVDKSRWQEGNVFSCSVMHEALHNHYTQKSLSLSLGK

SEQ ID NO: 75 - protein, 247 aa, synthetic construct
  REGION 1..247: note = amino acid sequence of antibody
QVQLVESGGGVVQPGRSLRLSCAASGFTFSSYTMHWVRQAPGKGLEWVTFISYDGNNKYYADSVKGRFTISRDNSKNTLYLQMNSLRAEDTAIYYCARTGWLGPFDYWGQGTLVTVSSGGGGSGGGGSGGGGSGGGGASEIVLTQSPGTLSLSPGERATLSCRASQSVGSSYLAWYQQKPGQAPRLLIYGAFSRATGIPDRFSGSGSGTDFTLTISRLEPEDFAVYYCQQYGSSPWTFGQGTKVEIK

SEQ ID NO: 76 - protein, 127 aa, synthetic construct
  REGION 1..127: note = amino acid sequence of antibody
QVQLVESGGGLVQPGGSLRLSCAASGYIYSAYCMGWFRQAPGKGLEGVAAIYIGGGSTYYADSVKGRFTISRDNSKNTLYLQMNSLRAEDTAVYYCAADVIPTETCLGGSWSGPFGYWGQGTLVTSS

SEQ ID NO: 77 - DNA, 24 bp, synthetic construct
  misc_feature 1..24: note = primer
  source 1..24: mol_type = other DNA
gtcctggctgctcttctacaaggc

SEQ ID NO: 78 - DNA, 23 bp, synthetic construct
  misc_feature 1..23: note = primer
  source 1..23: mol_type = other DNA
ggtacgtgctgttgaactgttcc

SEQ ID NO: 79 - DNA, 29 bp, synthetic construct
  misc_feature 1..29: note = primer
  source 1..29: mol_type = other DNA
gatgtgcagctgcaggagtctggrggagg

SEQ ID NO: 80 - DNA, 35 bp, synthetic construct
  misc_feature 1..35: note = primer
  source 1..35: mol_type = other DNA
ggactagtgcggccgctggagacggtgacctgggt